European Patent Specification EP 3 407 909 B1, published August 9, 2023. Title: Cancer treatment. Applicant: Propanc Pty Ltd. The sequence listing filed with the application follows.

SEQUENCE LISTING (22 sequences)

SEQ ID NO: 1 - DNA, 20 bp, Artificial Sequence
  SNAIL Forward primer
accccacatccttctcactg

SEQ ID NO: 2 - DNA, 20 bp, Artificial Sequence
  SNAIL Reverse primer
tacaaaaacccacgcagaca

SEQ ID NO: 3 - DNA, 20 bp, Artificial Sequence
  SLUG Forward primer
tgcgatgcccagtctagaaa

SEQ ID NO: 4 - DNA, 19 bp, Artificial Sequence
  SLUG Reverse primer
ttctcccccgtgtgagttc

SEQ ID NO: 5 - DNA, 20 bp, Artificial Sequence
  E-CADHERIN Forward primer
aattcctgccattctgggga

SEQ ID NO: 6 - DNA, 20 bp, Artificial Sequence
  E-CADHERIN Reverse primer
tcttctccgcctccttcttc

SEQ ID NO: 7 - DNA, 20 bp, Artificial Sequence
  N-CADHERIN Forward primer
tgagcctgaagccaacctta

SEQ ID NO: 8 - DNA, 20 bp, Artificial Sequence
  N-CADHERIN Reverse primer
aggtcccctggagttttctg

SEQ ID NO: 9 - DNA, 20 bp, Artificial Sequence
  VIMENTIN Forward primer
agctaaccaacgacaaagcc

SEQ ID NO: 10 - DNA, 20 bp, Artificial Sequence
  VIMENTIN Reverse primer
tccactttgcgttcaaggtc

SEQ ID NO: 11 - DNA, 20 bp, Artificial Sequence
  OCT4 Forward primer
caccatctgtcgcttcgagg

SEQ ID NO: 12 - DNA, 22 bp, Artificial Sequence
  OCT4 Reverse primer
agggtctccgatttgcatatct

SEQ ID NO: 13 - DNA, 20 bp, Artificial Sequence
  KLF4 Forward primer
cgaacccacacaggtgagaa

SEQ ID NO: 14 - DNA, 22 bp, Artificial Sequence
  KLF4 Reverse primer
tacggtagtgcctggtcagttc

SEQ ID NO: 15 - DNA, 20 bp, Artificial Sequence
  SOX 2 Forward primer
caagatgcacaactcgcaga

SEQ ID NO: 16 - DNA, 20 bp, Artificial Sequence
  SOX2 Reverse primer
catgagcgtcttggttttcc

SEQ ID NO: 17 - DNA, 21 bp, Artificial Sequence
  NANOG Forward primer
tcctgaacctcagctacaaac

SEQ ID NO: 18 - DNA, 20 bp, Artificial Sequence
  NANOG Reverse primer
gcgtcacaccattgctattc

SEQ ID NO: 19 - DNA, 22 bp, Artificial Sequence
  C-MYC Forward primer
gagtctggatcaccttctgctg

SEQ ID NO: 20 - DNA, 22 bp, Artificial Sequence
  C-MYC Reverse primer
aggatagtccttccgagtggag

SEQ ID NO: 21 - DNA, 21 bp, Artificial Sequence
  CD133 Forward primer
cagaataataaacagcagccc

SEQ ID NO: 22 - DNA, 21 bp, Artificial Sequence
  CD133 Reverse primer
gattatgacaagccagaaact